European Patent Application EP 4 427 761 A1, published September 11, 2024. Title: VACCINE AGAINST PANCREATIC CANCER, AND MEDICAL USE THEREOF. Applicant: YUANBAN (ZHUHAI HENGQIN) BIOTECHNOLOGY CO., LTD. The sequence listing filed with the application follows.

SEQUENCE LISTING (3 sequences)

SEQ ID NO: 1 - DNA, 420 bp, unidentified
  source 1..420: mol_type = other DNA
ggtgttacttctgctcctgatactcgtcctgctcctggttctactgcaccgccagcacatggcgtgacgtctgcgccagatacccgtccggcaccgggttccaccgccccaccggcacacggcgtaacctccgcgccagacacccgtccagcgccaggttctaccgctccgcctgctcatggtgttacctctgccccggacactcgtccggctccaggttctactgccccgccagctcatggcgtcacttccgccccggatacccgtcctgccccgggctctactgcgcctccggctcacggcgttacctctgcaccggatactcgtccggctccgggctctaccgcaccacctgctcatggcgtaacgagcgctcctgatacccgtccggctccgggttccactgcacctccggcccac

SEQ ID NO: 2 - DNA, 1164 bp, unidentified
  source 1..1164: mol_type = other DNA
aaaatcgaagaaggcaaactggtgatctggatcaacggtgataagggttataacggtctggcggaagtaggcaagaaattcgaaaaagacaccggtatcaaagttaccgttgaacatccagacaaactggaagaaaaattccctcaggtggcggctaccggcgacggccctgatatcattttctgggcacatgatcgttttggcggttacgcgcagtctggcctgctggcagaaatcacgccggataaggcgttccaggacaaactgtacccttttacctgggacgcggtgcgttacaacggcaaactgatcgcttacccgatcgcagtggaagctctgtccctgatctacaataaggacctgctgccgaacccgcctaaaacgtgggaagaaatcccggccctggacaaagaactgaaagcaaaaggtaagagcgctctgatgttcaatctgcaggaaccgtacttcacttggccgctgatcgcagctgacggcggttatgcgtttaaatacgaaaacggtaaatatgacattaaggacgtcggcgttgataacgccggcgccaaagcgggcctgacctttctggtcgacctgatcaaaaacaaacacatgaacgctgacaccgattattctattgcggaggcggcttttaacaagggcgagaccgcaatgaccatcaacggtccgtgggcttggtctaacatcgacacctccaaagtaaattacggtgttaccgtcctgccgaccttcaaaggtcaaccgagcaaaccgttcgtgggcgtgctgtccgcaggtatcaacgctgcctccccaaacaaagagctggccaaagagttcctggaaaactatctgctgaccgacgaaggcctggaagctgttaataaagacaaaccgctgggtgctgttgcactgaaatcctatgaagaagaactggtcaaagatccgcgtattgccgccactatggagaacgcgcagaaaggtgaaatcatgccgaacatcccgcaaatgtccgctttttggtacgcggtgcgtaccgctgtaattaacgcggcgtccggtcgtcagactgtcgatgaagcgctgaaagatgctcagactaactctagctctaacaataacaataataacaacaacaacaatctgggtattgaaggtcgcatctct

SEQ ID NO: 3 - protein, 528 aa, synthetic construct
KIEEGKLVIWINGDKGYNGLAEVGKKFEKDTGIKVTVEHPDKLEEKFPQVAATGDGPDIIFWAHDRFGGYAQSGLLAEITPDKAFQDKLYPFTWDAVRYNGKLIAYPIAVEALSLIYNKDLLPNPPKTWEEIPALDKELKAKGKSALMFNLQEPYFTWPLIAADGGYAFKYENGKYDIKDVGVDNAGAKAGLTFLVDLIKNKHMNADTDYSIAEAAFNKGETAMTINGPWAWSNIDTSKVNYGVTVLPTFKGQPSKPFVGVLSAGINAASPNKELAKEFLENYLLTDEGLEAVNKDKPLGAVALKSYEEELVKDPRIAATMENAQKGEIMPNIPQMSAFWYAVRTAVINAASGRQTVDEALKDAQTNSSSNNNNNNNNNNLGIEGRISGVTSAPDTRPAPGSTAPPAHGVTSAPDTRPAPGSTAPPAHGVTSAPDTRPAPGSTAPPAHGVTSAPDTRPAPGSTAPPAHGVTSAPDTRPAPGSTAPPAHGVTSAPDTRPAPGSTAPPAHGVTSAPDTRPAPGSTAPPAH